European Patent Application EP 4 810 627 A1, published September 23, 2026. Title: NEW TARGETS AND BIOMARKERS FOR THE PREVENTION AND TREATMENT OF SKIN AGEING. Applicant: L'OREAL. Application EP. The sequence listing filed with the application follows.

SEQUENCE LISTING (13 sequences)

SEQ ID NO: 1 - RNA, 22 nt, synthetic construct
  source 1..22: mol_type = other RNA
agccacaatcaccttctgatct

SEQ ID NO: 2 - DNA, 22 bp, synthetic construct
  source 1..22: mol_type = other DNA
agccacaatcaccttctgatct

SEQ ID NO: 3-4 - skipped (2 entries)

SEQ ID NO: 5 - DNA, 20 bp, synthetic construct
  source 1..20: mol_type = other DNA
cacaatcaccttctgatctg

SEQ ID NO: 6 - DNA, 20 bp, synthetic construct
  source 1..20: mol_type = other DNA
gacacttgctctttctgacc

SEQ ID NO: 7 - DNA, 20 bp, synthetic construct
  source 1..20: mol_type = other DNA
cgaactgacttcccagccga

SEQ ID NO: 8 - DNA, 20 bp, synthetic construct
  source 1..20: mol_type = other DNA
aggcacttacagaaaaggtg

SEQ ID NO: 9 - skipped

SEQ ID NO: 10 - DNA, 52 bp, synthetic construct
  source 1..52: mol_type = other DNA
gaattcagcatgtcctttgcaacgactagtcacaaatgatgaaaaagaatag

SEQ ID NO: 11 - DNA, 20 bp, synthetic construct
  source 1..20: mol_type = other DNA
aatgcagctggcacgacagg

SEQ ID NO: 12 - DNA, 20 bp, synthetic construct
  source 1..20: mol_type = other DNA
cctgtcgtgccagctgcatt

SEQ ID NO: 13 - DNA, 52 bp, synthetic construct
  source 1..52: mol_type = other DNA
ctattctttttcatcatttgtgactagtcgttgcaaaggacatgctgaattc